European Patent Application EP 4 768 472 A1, published July 1, 2026. Title: DRUG DELIVERY MATERIAL AND APPLICATION THEREOF. Applicant: DsciLab Co.,Ltd. The sequence listing filed with the application follows.

SEQUENCE LISTING (1 sequence)

SEQ ID NO: 1 - RNA, 1653 nt, synthetic construct
  source 1..1653: mol_type = other RNA
atggaggacgccaagaacatcaagaagggccccgcccccttctaccccctggaggacggcaccgccggcgagcagctgcacaaggccatgaagcggtacgccctggtgcccggcaccatcgccttcaccgacgcccacatcgaggtggacatcacctacgccgagtacttcgagatgagcgtgcggctggccgaggccatgaagcggtacggcctgaacaccaaccaccggatcgtggtgtgcagcgagaacagcctgcagttcttcatgcccgtgctgggcgccctgttcatcggcgtggccgtggcccccgccaacgacatctacaacgagcgggagctgctgaacagcatgggcatcagccagcccaccgtggtgttcgtgagcaagaagggcctgcagaagatcctgaacgtgcagaagaagctgcccatcatccagaagatcatcatcatggacagcaagaccgactaccagggcttccagagcatgtacaccttcgtgaccagccacctgccccccggcttcaacgagtacgacttcgtgcccgagagcttcgaccgggacaagaccatcgccctgatcatgaacagcagcggcagcaccggcctgcccaagggcgtggccctgccccaccggaccgcctgcgtgcggttcagccacgcccgggaccccatcttcggcaaccagatcatccccgacaccgccatcctgagcgtggtgcccttccaccacggcttcggcatgttcaccaccctgggctacctgatctgcggcttccgggtggtgctgatgtaccggttcgaggaggagctgttcctgcggagcctgcaggactacaagatccagagcgccctgctggtgcccaccctgttcagcttcttcgccaagagcaccctgatcgacaagtacgacctgagcaacctgcacgagatcgccagcggcggcgcccccctgagcaaggaggtgggcgaggccgtggccaagcggttccacctgcccggcatccggcagggctacggcctgaccgagaccaccagcgccatcctgatcacccccgagggcgacgacaagcccggcgccgtgggcaaggtggtgcccttcttcgaggccaaggtggtggacctggacaccggcaagaccctgggcgtgaaccagcggggcgagctgtgcgtgcggggccccatgatcatgagcggctacgtgaacaaccccgaggccaccaacgccctgatcgacaaggacggctggctgcacagcggcgacatcgcctactgggacgaggacgagcacttcttcatcgtggaccggctgaaaagcctgatcaagtacaagggctaccaggtggcccccgccgagctggagagcatcctgctgcagcaccccaacatcttcgacgccggcgtggccggcctgcccgacgacgacgccggcgagctgcccgccgccgtggtggtgctggagcacggcaagaccatgaccgagaaggagatcgtggactacgtggccagccaggtgaccaccgccaagaagctgcggggcggcgtggtgttcgtggacgaggtgcccaagggcctgaccggcaagctggacgcccggaagatccgggagatcctgatcaaggccaagaagggcggcaagatcgccgtgtga